European Patent Specification EP 3 818 155 B1, published September 6, 2023. Title: 3-Methylcrotonic acid decarboxylase (MDC) variants. Applicant: Global Bioenergies. The sequence listing filed with the application follows.

SEQUENCE LISTING (9 sequences)

SEQ ID NO: 1 - protein, 501 aa, Streptomyces sp. 769
MYVQMVFVKEVPVQHPSDLREHIEALEKLGDLDRVHDEVDWNLEAAAQTRYSTEHHLPAPLFENVAGVAEGFRLLGAPAALSSDPSRPYARVALSVGLRPEATGREVVEHLVAARHRPGVPPVAVAAEAAPVKANVLLGDEADLNRFPVPFVHEGDGNRYANTYGVIIAQTPDGSWTNWSIARIMMIDGKHMTGLVMHPQHIAQVWQQWADLGKPMPYALVQGGDPAIPYVGGIPIGDGVAESAYIGALIGRPLEVVKAELSDLMVPAGAEIVIEGHLSVQRDGVEGPFGEFAGYIPRETSLQPVYTVEAITHRDAPIWPLVAEGKPTDDFHTVTGIGEAAGALDAIREAGLPAASAWAPLSAASHWLVVTAPGNWRELLPGVSEEQYARRVGEAVFGTKFGSCLPQVFLLDDDFDPTDDADLLWALATRVHPDGRVVRFEDGPVLPLLTCYTPQERHAARATKVVHEALLSAPGEREPQSTFADAYPAEVRAKVRARYPN

SEQ ID NO: 2 - protein, 189 aa, Escherichia coli K-12
MKRLIVGISGASGAIYGVRLLQVLRDVTDIETHLVMSQAARQTLSLETDFSLREVQALADVTHDARDIAASISSGSFQTLGMVILPCSIKTLSGIVHSYTDGLLTRAADVVLKERRPLVLCVRETPLHLGHLRLMTQAAEIGAVIMPPVPAFYHRPQSLDDVINQTVNRVLDQFAITLPEDLFARWQGA

SEQ ID NO: 3 - protein, 229 aa, Candida albicans
  Candida albicans (strain SC5314 / ATCC MYA-2876)
MIARVCLRRSNVLPIFQIPSRKYSINYEKVNNSIYNNVIKPKRIVLAITGATGTQIGVRLLEILKELGVETHLVMSKWGIATLKYETDYQVDYVTSLATKTYSARDVTAPISSGSFVHDGMIVAPCSMKSLSAIRTGFTEDLIVRAADVSLKERRKLLLVARETPLSDIHLDNMLYLSRMGVTIFPPVPAFYTKPKTIDDIVEQTCGRILDNFGINIDTFERWDGINHR

SEQ ID NO: 4 - protein, 227 aa, Aspergillus niger
MFNSLLSGTTTPNSGRASPPASEMPIDNDHVAVARPAPRRRRIVVAMTGATGAMLGIKVLIALRRLNVETHLVMSKWAEATIKYETDYHPSNVRALADYVHNINDMAAPVSSGSFRADGMIVVPCSMKTLAAIHSGFCDDLISRTADVMLKERRRLVLVARETPLSEIHLRNMLEVTRAGAVIFPPVPAFYIKAGSIEDLIDQSVGRMLDLFDLDTGDFERWNGWEK

SEQ ID NO: 5 - protein, 242 aa, Saccharomyces cerevisiae S288c
MLLFPRRTNIAFFKTTGIFANFPLLGRTITTSPSFLTHKLSKEVTRASTSPPRPKRIVVAITGATGVALGIRLLQVLKELSVETHLVISKWGAATMKYETDWEPHDVAALATKTYSVRDVSACISSGSFQHDGMIVVPCSMKSLAAIRIGFTEDLITRAADVSIKENRKLLLVTRETPLSSIHLENMLSLCRAGVIIFPPVPAFYTRPKSLHDLLEQSVGRILDCFGIHADTFPRWEGIKSK

SEQ ID NO: 6 - protein, 180 aa, Cryptococcus gattii WM276
  serotype B
MRRKRYVVAVTGATGATLAIRLLQALRALDIETHLIISKWAVKTLKYETDMIERELKDLADYSYSNSDLAAPPSSGSFIHDGMFIIPCSMKTLAAVRIGLGDELISRSADVCLKEGRKLMLVVRETPLNDIHLENMLFLRRAGAIIFPPVPAYYIRPQTIDDLTNQTVGRILDSSKCSQK

SEQ ID NO: 7 - protein, 192 aa, Bacillus subtilis
MKLVIGMTGATGAIFGIRLLEYLKAAEIETHLVVSPWANVTITHETDYTLKDVEKLASYTYSHKDQAAAISSGSFETDGMIIAPCSMKSLASIRTGMADNLLTRAADVILKERKKLVLLTRETPLSQIHLENMLALTKMGSVILPPMPAFYNKPADMDELIDHIVFRTLDQFGIRLPEAKRWYGIEKQKGGI

SEQ ID NO: 8 - protein, 209 aa, Pseudomonas aeruginosa
MSGPERITLAMTGASGAQYGLRLLDCLVQEEREVHFLISKAAQLVMATETDVALPAKPQAMQAFLTEYCGAAAGQIRVFGQNDWMAPPASGSSAPNAMVICPCSTGTLSAVATGACNNLIERAADVALKERRPLVLVPREAPFSSIHLENMLKLSNLGAVILPAAPGFYHQPQSVEDLVDFVVARILNTLGIPQDMLPRWGEQHLVSDE

SEQ ID NO: 9 - protein, 219 aa, Enterobacter sp.
  Enterobacter sp. DC4
MLRQVRANALTCNSPQNPAQSALKSVRAKIMKRLIVGLSGASGAIYGVRLLQVLRNVAEVETHLVMSQAARQTLSLETDLSLRDVQALADVVHDARDIAASISSGSFKTAGMVILPCSIKTLSGIVNSYTDTLVTRAADVVLKERRPLVLCVRETPLHLGHLRLMTQAAELGAIIMPPVPAFYHRPTSLDDVINQTVNRVLDQFDIDLPEDLFTRWQGA